European Patent Specification EP 3 494 131 B1, published September 18, 2024. Title: IMPROVED METHODS FOR PRODUCING POLYNUCLEOTIDE LIBRARIES IN VACCINIA VIRUS/EUKARYOTIC CELLS. Applicant: Vaccinex, Inc. Smith, Ernest Shi, Shuying. The sequence listing filed with the application follows.

SEQUENCE LISTING (3 sequences)

SEQ ID NO: 1 - DNA, 1555 bp, Artificial Sequence
  Transfer Plasmid containing pVHE promoter
ggccaaaaattgaaaaactagatctatttattgcacgcggccgcaaaccatgggatggagctgtatcatcctcttcttggtagcaacagctacaggcgcgcatatggtcaccgtctcctcagggagtgcatccgccccaacccttttccccctcgtctcctgtgagaattccccgtcggatacgagcagcgtggccgttggctgcctcgcacaggacttccttcccgactccatcactttctcctggaaatacaagaacaactctgacatcagcagcacccggggcttcccatcagtcctgagagggggcaagtacgcagccacctcacaggtgctgctgccttccaaggacgtcatgcagggcacagacgaacacgtggtgtgcaaagtccagcaccccaacggcaacaaagaaaagaacgtgcctcttccagtgattgctgagctgcctcccaaagtgagcgtcttcgtcccaccccgcgacggcttcttcggcaacccccgcagcaagtccaagctcatctgccaggccacgggtttcagtccccggcagattcaggtgtcctggctgcgcgaggggaagcaggtggggtctggcgtcaccacggaccaggtgcaggctgaggccaaagagtctgggcccacgacctacaaggtgactagcacactgaccatcaaagagagcgactggctcagccagagcatgttcacctgccgcgtggatcacaggggcctgaccttccagcagaatgcgtcctccatgtgtgtccccgatcaagacacagccatccgggtcttcgccatccccccatcctttgccagcatcttcctcaccaagtccaccaagttgacctgcctggtcacagacctgaccacctatgacagcgtcaccatctcctggacccgccagaatggcgaagctgtgaaaacccacaccaacatctccgagagccaccccaatgccactttcagcgccgtgggtgaggccagcatctgcgaggatgactggaattccggggagaggttcacgtgcaccgtgacccacacagacctgccctcgccactgaagcagaccatctcccggcccaagggggtggccctgcacaggcccgatgtctacttgctgccaccagcccgggagcagctgaacctgcgggagtcggccaccatcacgtgcctggtgacgggcttctctcccgcggacgtcttcgtgcagtggatgcagagggggcagcccttgtccccggagaagtatgtgaccagcgccccaatgcctgagccccaggccccaggccggtacttcgcccacagcatcctgaccgtgtccgaagaggaatggaacacgggggagacctacacctgcgtggtggcccatgaggccctgcccaacagggtcactgagaggaccgtggacaagtccaccgagggggaggtgagcgccgacgaggagggctttgagaacctgtgggccaccgcctccaccttcatcgtcctcttcctcctgagcctcttctacagtaccaccgtcaccttgttcaaggtgaaatgagtcgac

SEQ ID NO: 2 - DNA, 446 bp, Artificial Sequence
  Transfer plasmid containing pVKE promoter
ggccaaaaattgaaaaactagatctatttattgcacgcggccgcccatgggatggagctgtatcatcctcttcttggtagcaacagctacacgggtgcacttgactcgagatcaaacgaactgtggctgcaccatctgtcttcatcttcccgccatctgatgagcagttgaaatctggaactgcctctgttgtgtgcctgctgaataacttctatcccagagaggccaaagtacagtggaaggtggataacgccctccaatcgggtaactcccaggagagtgtcacagagcaggacagcaaggacagcacctacagcctcagcagcaccctgacgctgagcaaagcagactacgagaaacacaaagtctacgcctgcgaagtcacccatcagggcctgagctcgcccgtcacaaagagcttcaacaggggagagtgttaggtcgac

SEQ ID NO: 3 - DNA, 455 bp, Artificial Sequence
  Transfer plasmid containing pVLE promoter
ggccaaaaattgaaaaactagatctatttattgcacgcggccgcccatgggatggagctgtatcatcctcttcttggtagcaacagctacaggcgtgcacttgactcgagaagcttaccgtcctacgaactgtggctgcaccatctgtcttcatcttcccgccatctgatgagcagttgaaatctggaactgcctctgttgtgtgcctgctgaataacttctatcccagagaggccaaagtacagtggaaggtggataacgccctccaatcgggtaactcccaggagagtgtcacagagcaggacagcaaggacagcacctacagcctcagcagcaccctgacgctgagcaaagcagactacgagaaacacaaagtctacgcctgcgaagtcacccatcagggcctgagctcgcccgtcacaaagagcttcaacaggggagagtgttaggtcgac